European Patent Specification EP 3 533 875 B1, published February 15, 2023. Title: CORYNEBACTERIUM FOR PRODUCING L-LYSINE BY FERMENTATION. Applicant: NINGXIA EPPEN BIOTECH CO.,LTD. The sequence listing filed with the application follows.

SEQUENCE LISTING (5 sequences)

SEQ ID NO: 1 - protein, 84 aa, Corynebacterium glutamicum
MSQARRYLVQDRGVSLSDADGVLVDLNFTCTQVNESNDTDDLSVFCSTAIAGKDPSELRKELEAEFYFLPDGADDADDADDAMG

SEQ ID NO: 2 - DNA, 255 bp, Corynebacterium glutamicum
ctagcccattgcatcgtctgcatcgtctgcatcgtctgcaccgtccggcaaaaaatagaattctgcttctagctctttccgtaattcggacggatcttttccagcgatggcggtactacagaaaacagatagatcatctgtgtcgttagactcattaacctgggtgcatgtgaaattgagatccactaaaacaccatcagcatcgctgagggaaacccctcgatcctggacaaggtatctgcgcgcttgagacat

SEQ ID NO: 3 - protein, 183 aa, Corynebacterium glutamicum
MKNAKLFLALISAPLILAGCSSTDTGTAESTISSETASAVDATTSTSSSTATSAVIDDDPVFDIIDIVLAQYPDRIITDIDREDSSDQYEVDVVVGQEVLELDVTTSGQIHTDDRDNDDDDDIREAHAATVTAAQAIGLALDQYPDGIIDSVELDEDDGQLKWKIDLDDTSGNDLADVEIAAV

SEQ ID NO: 4 - DNA, 552 bp, Corynebacterium glutamicum
ttaaactgctgcgatttcaacgtcagcaagatcattgccggaagtgtcatcgaggtctattttccatttcagctggccgtcgtcttcgtctaattcaacagaatcaataattccgtctgggtattgatccagcgctaggccaatggcttgagctgcggtgactgtggctgcgtgagcttcgcggatgtcgtcatcatcatcgttgtcgcggtcgtcggtatggatctggccactggtggtgacatcaagttcaaggacttcttggccaaccacaacatcgacttcgtattgatcggaggagtcttcgcggtcaatgtcggtgatgatcctgtcggggtattgggcaaggacgatgtcgatgatgtcgaataccggatcgtcatcaatcacggcagaggtggcggtacttgaggaggtagaagtggtggcatctactgcagaagcagtttcgctggaaatggtggattctgctgttccagtatcggtggagctgcagccagcgaggataagaggagcggatatgagcgcgaggaaaagttttgcgttcttcat

SEQ ID NO: 5 - DNA, 445 bp, Artificial Sequence
  Synthesized promoter
cgaggttaagtgtattttaggtgaacaaatttcagcttcgggtagaagaccttcgatgcgcttcagagcttctattgggaaatctgataccacttgattaaatagcctacccccgaattgggggattggtcattttttgctgtgaaggtagttttgatgcatatgacctgcgtttataaagaaatgtaaacgtgatcagatcgatataaaagaaacagtttgtactcaggtttgaagcattttctccgattcgcctggcaaaaatctcaattgtcgcttacagtttttctcaacgacaggctgctaagctgctagttcggtggcctagtgagtggcgtttacttggataaaagtaatcccatgtcgtgatcagccattttgggttgtttccatagcaatccaaaggtttcgtctttcgatacctattcaaggagccttcgcctct